European Patent Application EP 4 748 857 A1, published May 27, 2026. Title: Anti-CD40L/anti-CD28 bispecific antibody and use thereof. Applicant: Seoul National University R&DB Foundation. The sequence listing filed with the application follows.

SEQUENCE LISTING (128 sequences)

SEQ ID NO: 1 - protein, 13 aa, synthetic construct
  REGION 1..13: note = L-CDR1 of anti-CD40L antibody
SGGYSSYGIYYYG

SEQ ID NO: 2 - protein, 8 aa, synthetic construct
  REGION 1..8: note = L-CDR1 of anti-CD40L antibody
SGDSSWYG

SEQ ID NO: 3 - protein, 8 aa, synthetic construct
  REGION 1..8: note = L-CDR1 of anti-CD40L antibody
SGGSGSYG

SEQ ID NO: 4 - protein, 7 aa, synthetic construct
  REGION 1..7: note = L-CDR2 of anti-CD40L antibody
NGNKRPS

SEQ ID NO: 5 - protein, 7 aa, synthetic construct
  REGION 1..7: note = L-CDR2 of anti-CD40L antibody
ANTNRPS

SEQ ID NO: 6 - protein, 7 aa, synthetic construct
  REGION 1..7: note = L-CDR2 of anti-CD40L antibody
WDDERPS

SEQ ID NO: 7 - protein, 11 aa, synthetic construct
  REGION 1..11: note = L-CDR3 of anti-CD40L antibody
GSGDSSSDSGI

SEQ ID NO: 8 - protein, 10 aa, synthetic construct
  REGION 1..10: note = L-CDR3 of anti-CD40L antibody
GSADSTYTAA

SEQ ID NO: 9 - protein, 11 aa, synthetic construct
  REGION 1..11: note = L-CDR3 of anti-CD40L antibody
GGYDDSSYAGI

SEQ ID NO: 10 - protein, 10 aa, synthetic construct
  REGION 1..10: note = H-CDR1 of anti-CD40L antibody
GFTFSSYGMN

SEQ ID NO: 11 - protein, 10 aa, synthetic construct
  REGION 1..10: note = H-CDR1 of anti-CD40L antibody
GFDFSSYDMN

SEQ ID NO: 12 - protein, 10 aa, synthetic construct
  REGION 1..10: note = H-CDR1 of anti-CD40L antibody
GFTFSSYGMQ

SEQ ID NO: 13 - protein, 17 aa, synthetic construct
  REGION 1..17: note = H-CDR2 of anti-CD40L antibody
AISNDGSSTSYAPAVKG

SEQ ID NO: 14 - protein, 17 aa, synthetic construct
  REGION 1..17: note = H-CDR2 of anti-CD40L antibody
GIYDDGSGTVYAPAVKG

SEQ ID NO: 15 - protein, 17 aa, synthetic construct
  REGION 1..17: note = H-CDR2 of anti-CD40L antibody
AIDDDGSSTNYGAAVKG

SEQ ID NO: 16 - protein, 14 aa, synthetic construct
  REGION 1..14: note = H-CDR3 of anti-CD40L antibody
ESTNGGWVADDIDA

SEQ ID NO: 17 - protein, 9 aa, synthetic construct
  REGION 1..9: note = H-CDR3 of anti-CD40L antibody
GGGADNIDA

SEQ ID NO: 18 - protein, 16 aa, synthetic construct
  REGION 1..16: note = H-CDR3 of anti-CD40L antibody
DGIIYYWNADAGYIDA

SEQ ID NO: 19 - protein, 20 aa, synthetic construct
  REGION 1..20: note = L-FR1 of anti-CD40L antibody
ALTQPSSVSANLGGTVKITC

SEQ ID NO: 20 - protein, 20 aa, synthetic construct
  REGION 1..20: note = L-FR1 of anti-CD40L antibody
ELTQDPAVSVALGQTVRITC

SEQ ID NO: 21 - protein, 19 aa, synthetic construct
  REGION 1..19: note = L-FR1 of anti-CD40L antibody
LTQASSVSANLGGTVEITC

SEQ ID NO: 22 - protein, 19 aa, synthetic construct
  REGION 1..19: note = L-FR1 of anti-CD40L antibody
LTQPSSVSANPGETVKITC

SEQ ID NO: 23 - protein, 16 aa, synthetic construct
  REGION 1..16: note = L-FR2 of anti-CD40L antibody
WYQQKSPGSAPVTLIY

SEQ ID NO: 24 - protein, 15 aa, synthetic construct
  REGION 1..15: note = L-FR2 of anti-CD40L antibody
WYQQKPGQAPVTVIY

SEQ ID NO: 25 - protein, 32 aa, synthetic construct
  REGION 1..32: note = L-FR3 of anti-CD40L antibody
NIPSRFSGSTSGSTNTLTITGVQVDDEAVYFC

SEQ ID NO: 26 - protein, 32 aa, synthetic construct
  REGION 1..32: note = L-FR3 of anti-CD40L antibody
GIPDRFSGSSSGNTASLTITGAQAEDEADYYC

SEQ ID NO: 27 - protein, 32 aa, synthetic construct
  REGION 1..32: note = L-FR3 of anti-CD40L antibody
DIPSRFSGSTSGSTGTLTITGVQADDEAVYYC

SEQ ID NO: 28 - protein, 32 aa, synthetic construct
  REGION 1..32: note = L-FR3 of anti-CD40L antibody
DIPSRFSGSKSGSTATLTITGVQAEDEAVYFC

SEQ ID NO: 29 - protein, 10 aa, synthetic construct
  REGION 1..10: note = L-FR4 of anti-CD40L antibody
FGAGTTLTVL

SEQ ID NO: 30 - protein, 10 aa, synthetic construct
  REGION 1..10: note = L-FR4 of anti-CD40L antibody
FGGGTKLTVL

SEQ ID NO: 31 - protein, 10 aa, synthetic construct
  REGION 1..10: note = L-FR4 of anti-CD40L antibody
FGAGTTLTVL

SEQ ID NO: 32 - protein, 25 aa, synthetic construct
  REGION 1..25: note = H-FR1 of anti-CD40L antibody
AVTLDESGGGLQTPGGALSLVCKAS

SEQ ID NO: 33 - protein, 25 aa, synthetic construct [sequence omitted]

SEQ ID NO: 34 - protein, 25 aa, synthetic construct
  REGION 1..25: note = H-FR1 of anti-CD40L antibody
EVQLVESGGGLVQPGGSLRLICAAS

SEQ ID NO: 35 - protein, 25 aa, synthetic construct
  REGION 1..25: note = H-FR1 of anti-CD40L antibody
AVTLDESGGGLQTPGGTLSLVCKAS

SEQ ID NO: 36 - protein, 25 aa, synthetic construct
  REGION 1..25: note = H-FR1 of anti-CD40L antibody
AVTLDESGGGLHTPGGALSLVCKAS

SEQ ID NO: 37 - protein, 14 aa, synthetic construct
  REGION 1..14: note = H-FR2 of anti-CD40L antibody
WVRQAPGKGLEWVG

SEQ ID NO: 38 - protein, 14 aa, synthetic construct
  REGION 1..14: note = H-FR2 of anti-CD40L antibody
WVRQAPGKGLEWVS

SEQ ID NO: 39 - protein, 14 aa, synthetic construct
  REGION 1..14: note = H-FR2 of anti-CD40L antibody
WVRQAPGKGLEYVA

SEQ ID NO: 40 - protein, 14 aa, synthetic construct
  REGION 1..14: note = H-FR2 of anti-CD40L antibody
WVRQAPGKGLEFVA

SEQ ID NO: 41 - protein, 32 aa, synthetic construct
  REGION 1..32: note = H-FR3 of anti-CD40L antibody
RATISRDNGQSTVRLQLNNLRAEDTATYYCAK

SEQ ID NO: 42 - protein, 32 aa, synthetic construct
  REGION 1..32: note = H-FR3 of anti-CD40L antibody
RFTISRDNSKNTLYLQMNSLRAEDTAVYYCAK

SEQ ID NO: 43 - protein, 32 aa, synthetic construct
  REGION 1..32: note = H-FR3 of anti-CD40L antibody
RATISRDNGQSTVRLQLNNLRAEDTGTYYCTR

SEQ ID NO: 44 - protein, 32 aa, synthetic construct
  REGION 1..32: note = H-FR3 of anti-CD40L antibody
RATISRDNGQSTVRLQLNNLRAEDTGTYYCAK

SEQ ID NO: 45 - protein, 11 aa, synthetic construct
  REGION 1..11: note = H-FR4 of anti-CD40L antibody
WGHGTEVIVSS

SEQ ID NO: 46 - protein, 11 aa, synthetic construct
  REGION 1..11: note = H-FR4 of anti-CD40L antibody
WGQGTLVTVSS

SEQ ID NO: 47 - protein, 109 aa, synthetic construct
  REGION 1..109: note = VL of anti-CD40L antibody
ALTQPSSVSANLGGTVKITCSGGYSSYGIYYYGWYQQKSPGSAPVTLIYNGNKRPSNIPSRFSGSTSGSTNTLTITGVQVDDEAVYFCGSGDSSSDSGIFGAGTTLTVL

SEQ ID NO: 48 - protein, 108 aa, synthetic construct
  REGION 1..108: note = VL of anti-CD40L antibody
ELTQDPAVSVALGQTVRITCSGGYSSYGIYYYGWYQQKPGQAPVTVIYNGNKRPSGIPDRFSGSSSGNTASLTITGAQAEDEADYYCGSGDSSSDSGIFGGGTKLTVL

SEQ ID NO: 49 - protein, 102 aa, synthetic construct
  REGION 1..102: note = VL of anti-CD40L antibody
LTQASSVSANLGGTVEITCSGDSSWYGWYQQKSPGSAPVTLIYANTNRPSDIPSRFSGSTSGSTGTLTITGVQADDEAVYYCGSADSTYTAAFGAGTTLTVL

SEQ ID NO: 50 - protein, 103 aa, synthetic construct
  REGION 1..103: note = VL of anti-CD40L antibody
LTQPSSVSANPGETVKITCSGGSGSYGWYQQKSPGSAPVTLIYWDDERPSDIPSRFSGSKSGSTATLTITGVQAEDEAVYFCGGYDDSSYAGIFGAGTTLTVL

SEQ ID NO: 51 - protein, 123 aa, synthetic construct
  REGION 1..123: note = VH of anti-CD40L antibody
AVTLDESGGGLQTPGGALSLVCKASGFTFSSYGMNWVRQAPGKGLEWVGAISNDGSSTSYAPAVKGRATISRDNGQSTVRLQLNNLRAEDTATYYCAKESTNGGWVADDIDAWGHGTEVIVSS

SEQ ID NO: 52 - protein, 123 aa, synthetic construct
  REGION 1..123: note = VH of anti-CD40L antibody
EVQLVESGGGLVQPGGSLRLSCAASGFTFSSYGMNWVRQAPGKGLEWVSAISNDGSSTSYAPAVKGRFTISRDNSKNTLYLQMNSLRAEDTAVYYCAKESTNGGWVADDIDAWGQGTLVTVSS

SEQ ID NO: 53 - protein, 123 aa, synthetic construct
  REGION 1..123: note = VH of anti-CD40L antibody
EVQLVESGGGLVQPGGSLRLSCAASGFTFSSYGMNWVRQAPGKGLEWVGAISNDGSSTSYAPAVKGRFTISRDNSKNTLYLQMNSLRAEDTAVYYCAKESTNGGWVADDIDAWGQGTLVTVSS

SEQ ID NO: 54 - protein, 123 aa, synthetic construct
  REGION 1..123: note = VH of anti-CD40L antibody
EVQLVESGGGLVQPGGSLRLICAASGFTFSSYGMNWVRQAPGKGLEWVSAISNDGSSTSYAPAVKGRFTISRDNSKNTLYLQMNSLRAEDTAVYYCAKESTNGGWVADDIDAWGQGTLVTVSS

SEQ ID NO: 55 - protein, 123 aa, synthetic construct
  REGION 1..123: note = VH of anti-CD40L antibody
EVQLVESGGGLVQPGGSLRLICAASGFTFSSYGMNWVRQAPGKGLEWVGAISNDGSSTSYAPAVKGRFTISRDNSKNTLYLQMNSLRAEDTAVYYCAKESTNGGWVADDIDAWGQGTLVTVSS

SEQ ID NO: 56 - protein, 118 aa, synthetic construct
  REGION 1..118: note = VH of anti-CD40L antibody
AVTLDESGGGLQTPGGTLSLVCKASGFDFSSYDMNWVRQAPGKGLEYVAGIYDDGSGTVYAPAVKGRATISRDNGQSTVRLQLNNLRAEDTGTYYCTRGGGADNIDAWGHGTEVIVSS

SEQ ID NO: 57 - protein, 125 aa, synthetic construct
  REGION 1..125: note = VH of anti-CD40L antibody
AVTLDESGGGLHTPGGALSLVCKASGFTFSSYGMQWVRQAPGKGLEFVAAIDDDGSSTNYGAAVKGRATISRDNGQSTVRLQLNNLRAEDTGTYYCAKDGIIYYWNADAGYIDAWGHGTEVIVSS

SEQ ID NO: 58 - protein, 250 aa, synthetic construct
  REGION 1..250: note = scFv of anti-CD40L antibody
ALTQPSSVSANLGGTVKITCSGGYSSYGIYYYGWYQQKSPGSAPVTLIYNGNKRPSNIPSRFSGSTSGSTNTLTITGVQVDDEAVYFCGSGDSSSDSGIFGAGTTLTVLGQSSRSSGGGGSSGGGGSAVTLDESGGGLQTPGGALSLVCKASGFTFSSYGMNWVRQAPGKGLEWVGAISNDGSSTSYAPAVKGRATISRDNGQSTVRLQLNNLRAEDTATYYCAKESTNGGWVADDIDAWGHGTEVIVSS

SEQ ID NO: 59 - protein, 249 aa, synthetic construct
  REGION 1..249: note = scFv of anti-CD40L antibody
ELTQDPAVSVALGQTVRITCSGGYSSYGIYYYGWYQQKPGQAPVTVIYNGNKRPSGIPDRFSGSSSGNTASLTITGAQAEDEADYYCGSGDSSSDSGIFGGGTKLTVLGQSSRSSGGGGSSGGGGSEVQLVESGGGLVQPGGSLRLSCAASGFTFSSYGMNWVRQAPGKGLEWVSAISNDGSSTSYAPAVKGRFTISRDNSKNTLYLQMNSLRAEDTAVYYCAKESTNGGWVADDIDAWGQGTLVTVSS

SEQ ID NO: 60 - protein, 249 aa, synthetic construct
  REGION 1..249: note = scFv of anti-CD40L antibody
ELTQDPAVSVALGQTVRITCSGGYSSYGIYYYGWYQQKPGQAPVTVIYNGNKRPSGIPDRFSGSSSGNTASLTITGAQAEDEADYYCGSGDSSSDSGIFGGGTKLTVLGQSSRSSGGGGSSGGGGSEVQLVESGGGLVQPGGSLRLSCAASGFTFSSYGMNWVRQAPGKGLEWVGAISNDGSSTSYAPAVKGRFTISRDNSKNTLYLQMNSLRAEDTAVYYCAKESTNGGWVADDIDAWGQGTLVTVSS

SEQ ID NO: 61 - protein, 249 aa, synthetic construct
  REGION 1..249: note = scFv of anti-CD40L antibody
ELTQDPAVSVALGQTVRITCSGGYSSYGIYYYGWYQQKPGQAPVTVIYNGNKRPSGIPDRFSGSSSGNTASLTITGAQAEDEADYYCGSGDSSSDSGIFGGGTKLTVLGQSSRSSGGGGSSGGGGSEVQLVESGGGLVQPGGSLRLICAASGFTFSSYGMNWVRQAPGKGLEWVSAISNDGSSTSYAPAVKGRFTISRDNSKNTLYLQMNSLRAEDTAVYYCAKESTNGGWVADDIDAWGQGTLVTVSS

SEQ ID NO: 62 - protein, 249 aa, synthetic construct
  REGION 1..249: note = scFv of anti-CD40L antibody
ELTQDPAVSVALGQTVRITCSGGYSSYGIYYYGWYQQKPGQAPVTVIYNGNKRPSGIPDRFSGSSSGNTASLTITGAQAEDEADYYCGSGDSSSDSGIFGGGTKLTVLGQSSRSSGGGGSSGGGGSEVQLVESGGGLVQPGGSLRLICAASGFTFSSYGMNWVRQAPGKGLEWVGAISNDGSSTSYAPAVKGRFTISRDNSKNTLYLQMNSLRAEDTAVYYCAKESTNGGWVADDIDAWGQGTLVTVSS

SEQ ID NO: 63 - protein, 238 aa, synthetic construct
  REGION 1..238: note = scFv of anti-CD40L antibody
LTQASSVSANLGGTVEITCSGDSSWYGWYQQKSPGSAPVTLIYANTNRPSDIPSRFSGSTSGSTGTLTITGVQADDEAVYYCGSADSTYTAAFGAGTTLTVLGQSSRSSGGGGSSGGGGSAVTLDESGGGLQTPGGTLSLVCKASGFDFSSYDMNWVRQAPGKGLEYVAGIYDDGSGTVYAPAVKGRATISRDNGQSTVRLQLNNLRAEDTGTYYCTRGGGADNIDAWGHGTEVIVSS

SEQ ID NO: 64 - protein, 246 aa, synthetic construct
  REGION 1..246: note = scFv of anti-CD40L antibody
LTQPSSVSANPGETVKITCSGGSGSYGWYQQKSPGSAPVTLIYWDDERPSDIPSRFSGSKSGSTATLTITGVQAEDEAVYFCGGYDDSSYAGIFGAGTTLTVLGQSSRSSGGGGSSGGGGSAVTLDESGGGLHTPGGALSLVCKASGFTFSSYGMQWVRQAPGKGLEFVAAIDDDGSSTNYGAAVKGRATISRDNGQSTVRLQLNNLRAEDTGTYYCAKDGIIYYWNADAGYIDAWGHGTEVIVSS

SEQ ID NO: 65 - protein, 9 aa, synthetic construct
  REGION 1..9: note = L-CDR1 of anti-CD28 antibody
SGGGSNNYG

SEQ ID NO: 66 - protein, 7 aa, synthetic construct
  REGION 1..7: note = L-CDR2 of anti-CD28 antibody
YNDKRPS

SEQ ID NO: 67 - protein, 10 aa, synthetic construct
  REGION 1..10: note = L-CDR3 of anti-CD28 antibody
GSRDSSHDGI

SEQ ID NO: 68 - protein, 10 aa, synthetic construct
  REGION 1..10: note = H-CDR1 of anti-CD28 antibody
GFTFSTFNMF

SEQ ID NO: 69 - protein, 10 aa, synthetic construct
  REGION 1..10: note = H-CDR1 of anti-CD28 antibody
GFTFSSYAMH

SEQ ID NO: 70 - protein, 18 aa, synthetic construct
  REGION 1..18: note = H-CDR2 of anti-CD28 antibody
QISSNDGSWTGYGAAVKG

SEQ ID NO: 71 - protein, 19 aa, synthetic construct
  REGION 1..19: note = H-CDR3 of anti-CD28 antibody
AAGGYNVCGYGCGGDYIDA

SEQ ID NO: 72 - protein, 19 aa, synthetic construct
  REGION 1..19: note = L-FR1 of anti-CD28 antibody
MTQPSSVSANPGETVKITC

SEQ ID NO: 73 - protein, 19 aa, synthetic construct
  REGION 1..19: note = L-FR1 of anti-CD28 antibody
LTQPSSVSANPGETVKITC

SEQ ID NO: 74 - protein, 16 aa, synthetic construct
  REGION 1..16: note = L-FR2 of anti-CD28 antibody
WYQQKSPGSAPVTVIY

SEQ ID NO: 75 - protein, 15 aa, synthetic construct
  REGION 1..15: note = L-FR2 of anti-CD28 antibody
WYQQKPGSAPVTVIY

SEQ ID NO: 76 - protein, 32 aa, synthetic construct
  REGION 1..32: note = L-FR3 of anti-CD28 antibody
GIPSRFSGSTSGSTGTLTITGVRAEDEAVYFC

SEQ ID NO: 77 - protein, 10 aa, synthetic construct
  REGION 1..10: note = L-FR4 of anti-CD28 antibody
FGAGTTLTVL

SEQ ID NO: 78 - protein, 10 aa, synthetic construct
  REGION 1..10: note = L-FR4 of anti-CD28 antibody
FGGGTKLTVL

SEQ ID NO: 79 - protein, 25 aa, synthetic construct
  REGION 1..25: note = H-FR1 of anti-CD28 antibody
AVTLDESGGGLQTPGGALSLVCKAS

SEQ ID NO: 80 - protein, 25 aa, synthetic construct
  REGION 1..25: note = H-FR1 of anti-CD28 antibody
PVKLVESGGGLVTPGGSLRLSCSAS

SEQ ID NO: 81 - protein, 14 aa, synthetic construct
  REGION 1..14: note = H-FR2 of anti-CD28 antibody
WVRQAPGKGLEYVA

SEQ ID NO: 82 - protein, 14 aa, synthetic construct
  REGION 1..14: note = H-FR2 of anti-CD28 antibody
WVRQAPGKGLEYVG

SEQ ID NO: 83 - protein, 32 aa, synthetic construct; identical to SEQ ID NO: 41
  REGION 1..32: note = H-FR3 of anti-CD28 antibody

SEQ ID NO: 84 - protein, 32 aa, synthetic construct
  REGION 1..32: note = H-FR3 of anti-CD28 antibody
RFTISRDNSKSTLYLQMNSLRAEDTAVYYCAK

SEQ ID NO: 85 - protein, 13 aa, synthetic construct
  REGION 1..13: note = H-FR4 of anti-CD28 antibody
WGHGTEVIVSSTS

SEQ ID NO: 86 - protein, 13 aa, synthetic construct
  REGION 1..13: note = H-FR4 of anti-CD28 antibody
WGHGTQVTVSSTS

SEQ ID NO: 87 - protein, 103 aa, synthetic construct
  REGION 1..103: note = VL of anti-CD28 antibody
MTQPSSVSANPGETVKITCSGGGSNNYGWYQQKSPGSAPVTVIYYNDKRPSGIPSRFSGSTSGSTGTLTITGVRAEDEAVYFCGSRDSSHDGIFGAGTTLTVL

SEQ ID NO: 88 - protein, 102 aa, synthetic construct
  REGION 1..102: note = VL of anti-CD28 antibody
LTQPSSVSANPGETVKITCSGGGSNNYGWYQQKPGSAPVTVIYYNDKRPSGIPSRFSGSTSGSTGTLTITGVRAEDEAVYFCGSRDSSHDGIFGGGTKLTVL

SEQ ID NO: 89 - protein, 131 aa, synthetic construct
  REGION 1..131: note = VH of anti-CD28 antibody
AVTLDESGGGLQTPGGALSLVCKASGFTFSTFNMFWVRQAPGKGLEYVAQISSNDGSWTGYGAAVKGRATISRDNGQSTVRLQLNNLRAEDTATYYCAKAAGGYNVCGYGCGGDYIDAWGHGTEVIVSSTS

SEQ ID NO: 90 - protein, 131 aa, synthetic construct
  REGION 1..131: note = VH of anti-CD28 antibody
PVKLVESGGGLVTPGGSLRLSCSASGFTFSSYAMHWVRQAPGKGLEYVGQISSNDGSWTGYGAAVKGRFTISRDNSKSTLYLQMNSLRAEDTAVYYCAKAAGGYNVCGYGCGGDYIDAWGHGTQVTVSSTS

SEQ ID NO: 91 - protein, 252 aa, synthetic construct
  REGION 1..252: note = scFv of anti-CD28 antibody
MTQPSSVSANPGETVKITCSGGGSNNYGWYQQKSPGSAPVTVIYYNDKRPSGIPSRFSGSTSGSTGTLTITGVRAEDEAVYFCGSRDSSHDGIFGAGTTLTVLGQSSRSSGGGGSSGGGGSAVTLDESGGGLQTPGGALSLVCKASGFTFSTFNMFWVRQAPGKGLEYVAQISSNDGSWTGYGAAVKGRATISRDNGQSTVRLQLNNLRAEDTATYYCAKAAGGYNVCGYGCGGDYIDAWGHGTEVIVSSTS

SEQ ID NO: 92 - protein, 251 aa, synthetic construct
  REGION 1..251: note = scFv of anti-CD28 antibody
LTQPSSVSANPGETVKITCSGGGSNNYGWYQQKPGSAPVTVIYYNDKRPSGIPSRFSGSTSGSTGTLTITGVRAEDEAVYFCGSRDSSHDGIFGGGTKLTVLGQSSRSSGGGGSSGGGGSPVKLVESGGGLVTPGGSLRLSCSASGFTFSSYAMHWVRQAPGKGLEYVGQISSNDGSWTGYGAAVKGRFTISRDNSKSTLYLQMNSLRAEDTAVYYCAKAAGGYNVCGYGCGGDYIDAWGHGTQVTVSSTS

SEQ ID NO: 93 - protein, 18 aa, synthetic construct
  REGION 1..18: note = peptide linker
GQSSRSSGGGGSSGGGGS

SEQ ID NO: 94 - protein, 15 aa, synthetic construct
  REGION 1..15: note = peptide linker
GGGGSGGGGSGGGGS

SEQ ID NO: 95 - protein, 107 aa, synthetic construct
  REGION 1..107: note = Constant region of IgG Kappa
RTVAAPSVFIFPPSDEQLKSGTASVVCLLNNFYPREAKVQWKVDNALQSGNSQESVTEQDSKDSTYSLSSTLTLSKADYEKHKVYACEVTHQGLSLPVTKSFNRGES

SEQ ID NO: 96 - protein, 648 aa, synthetic construct
  REGION 1..648: note = anti-CD40L/anti-CD28 bispecific antibody
ELTQDPAVSVALGQTVRITCSGGYSSYGIYYYGWYQQKPGQAPVTVIYNGNKRPSGIPDRFSGSSSGNTASLTITGAQAEDEADYYCGSGDSSSDSGIFGGGTKLTVLGQSSRSSGGGGSSGGGGSEVQLVESGGGLVQPGGSLRLSCAASGFTFSSYGMNWVRQAPGKGLEWVGAISNDGSSTSYAPAVKGRFTISRDNSKNTLYLQMNSLRAEDTAVYYCAKESTNGGWVADDIDAWGQGTLVTVSSGQAGQGGGGSGGGGSGGGGSKLRTVAAPSVFIFPPSDEQLKSGTASVVCLLNNFYPREAKVQWKVDNALQSGNSQESVTEQDSKDSTYSLSSTLTLSKADYEKHKVYACEVTHQGLSLPVTKSFNRGESLEGGGGSGGGGSGGGGSTGLTQPSSVSANPGETVKITCSGGGSNNYGWYQQKPGSAPVTVIYYNDKRPSGIPSRFSGSTSGSTGTLTITGVRAEDEAVYFCGSRDSSHDGIFGGGTKLTVLGQSSRSSGGGGSSGGGGSPVKLVESGGGLVTPGGSLRLSCSASGFTFSSYAMHWVRQAPGKGLEYVGQISSNDGSWTGYGAAVKGRFTISRDNSKSTLYLQMNSLRAEDTAVYYCAKAAGGYNVCGYGCGGDYIDAWGHGTQVTVSSTS

SEQ ID NO: 97 - protein, 648 aa, synthetic construct
  REGION 1..648: note = anti-CD40L/anti-CD28 bispecific antibody
LTQPSSVSANPGETVKITCSGGGSNNYGWYQQKPGSAPVTVIYYNDKRPSGIPSRFSGSTSGSTGTLTITGVRAEDEAVYFCGSRDSSHDGIFGGGTKLTVLGQSSRSSGGGGSSGGGGSPVKLVESGGGLVTPGGSLRLSCSASGFTFSSYAMHWVRQAPGKGLEYVGQISSNDGSWTGYGAAVKGRFTISRDNSKSTLYLQMNSLRAEDTAVYYCAKAAGGYNVCGYGCGGDYIDAWGHGTQVTVSSTSGQAGQGGGGSGGGGSGGGGSKLRTVAAPSVFIFPPSDEQLKSGTASVVCLLNNFYPREAKVQWKVDNALQSGNSQESVTEQDSKDSTYSLSSTLTLSKADYEKHKVYACEVTHQGLSLPVTKSFNRGESLEGGGGSGGGGSGGGGSTGELTQDPAVSVALGQTVRITCSGGYSSYGIYYYGWYQQKPGQAPVTVIYNGNKRPSGIPDRFSGSSSGNTASLTITGAQAEDEADYYCGSGDSSSDSGIFGGGTKLTVLGQSSRSSGGGGSSGGGGSEVQLVESGGGLVQPGGSLRLSCAASGFTFSSYGMNWVRQAPGKGLEWVGAISNDGSSTSYAPAVKGRFTISRDNSKNTLYLQMNSLRAEDTAVYYCAKESTNGGWVADDIDAWGQGTLVTVSS

SEQ ID NO: 98 - protein, 102 aa, synthetic construct
  REGION 1..102: note = VL of anti-CD28 antibody
LTQPSSVSVSPGQTARITCSGGGSNNYGWYQQKPGSAPVTVIYYNDKRPSGIPERFSGSTSGSTGTLTISGVQAEDEAVYFCGSRDSSHDGIFGGGTKLTVL

SEQ ID NO: 99 - protein, 131 aa, synthetic construct
  REGION 1..131: note = VH of anti-CD28 antibody
EVQLVESGGGLVQPGGSLRLSCSASGFTFSSYAMHWVRQAPGKGLEYVGQISSNDGSWTGYGAAVKGRFTISRDNSKSTLYLQMNSLRAEDTAVYYCAKAAGGYNVCGYGCGGDYIDAWGQGTLVTVSSTS

SEQ ID NO: 100 - protein, 102 aa, synthetic construct
  REGION 1..102: note = VL of anti-CD28 antibody
LTQPSSVSVSPGQTARITCSGGGSNNYGWYQQKPGQAPVTVIYYNDKRPSGIPERFSGSTSGSTGTLTISGVQAEDEAVYFCGSRDSSHDGIFGGGTKLTVL

SEQ ID NO: 101 - protein, 131 aa, synthetic construct
  REGION 1..131: note = VH of anti-CD28 antibody
EVQLVESGGGLVQPGGSLRLSCSASGFTFSSYAMHWVRQAPGKGLEYVGQISSNDGSWTGYGAAVKGRFTISRDNSKNTLYLQMNSLRAEDTAVYYCAKAAGGYNVCGYGCGGDYIDAWGQGTLVTVSSTS

SEQ ID NO: 102 - protein, 17 aa, synthetic construct
  REGION 1..17: note = L-CDR1 of anti-CD28 antibody (mouse)
RSSQSLYYSGIKKNLLA

SEQ ID NO: 103 - protein, 7 aa, synthetic construct
  REGION 1..7: note = L-CDR2 of anti-CD28 antibody (mouse)
FTSTRLP

SEQ ID NO: 104 - protein, 9 aa, synthetic construct
  REGION 1..9: note = L-CDR3 of anti-CD28 antibody (mouse)
QQGISTPLT

SEQ ID NO: 105 - protein, 5 aa, synthetic construct
  REGION 1..5: note = H-CDR1 of anti-CD28 antibody (mouse)
DGYMN

SEQ ID NO: 106 - protein, 17 aa, synthetic construct
  REGION 1..17: note = H-CDR2 of anti-CD28 antibody (mouse)
RIDPDSGNTRYNQKFQG

SEQ ID NO: 107 - protein, 15 aa, synthetic construct
  REGION 1..15: note = H-CDR3 of anti-CD28 antibody (mouse)
DGTFYGTYGYWYFDF

SEQ ID NO: 108 - protein, 113 aa, synthetic construct
  REGION 1..113: note = VL of anti-CD28 antibody (mouse)
DIVMTQSPYSLAVSAGEKVTMSCRSSQSLYYSGIKKNLLAWYQQKPGQSPKLLIYFTSTRLPGVPDRFTGSGSGTDYTLTITSVQAEDMGHYFCQQGISTPLTFGDGTKLEIR

SEQ ID NO: 109 - protein, 124 aa, synthetic construct
  REGION 1..124: note = VH of anti-CD28 antibody (mouse)
QVQLKQSGAELVKPGASVKISCKTSGYTFTDGYMNWVEQKPGQGLEWIGRIDPDSGNTRYNQKFQGKATLTRDKSSSTVYMDLRSLTSEDSAVYYCARDGTFYGTYGYWYFDFWGQGTQVTVSS

SEQ ID NO: 110 - protein, 9 aa, synthetic construct
  REGION 1..9: note = L-CDR1 of anti-CD40L antibody (mouse)
SGGYSDYYG

SEQ ID NO: 111 - protein, 7 aa, synthetic construct
  REGION 1..7: note = L-CDR2 of anti-CD40L antibody (mouse)
YNDKRPS

SEQ ID NO: 112 - protein, 11 aa, synthetic construct
  REGION 1..11: note = L-CDR3 of anti-CD40L antibody (mouse)
GGYDGSTDAGI

SEQ ID NO: 113 - protein, 10 aa, synthetic construct
  REGION 1..10: note = H-CDR1 of anti-CD40L antibody (mouse)
GFTFNNNGMA

SEQ ID NO: 114 - protein, 16 aa, synthetic construct
  REGION 1..16: note = H-CDR2 of anti-CD40L antibody (mouse)
GISSGSYTYYGTAVKG

SEQ ID NO: 115 - protein, 16 aa, synthetic construct
  REGION 1..16: note = H-CDR3 of anti-CD40L antibody (mouse)
DGSDYNWNSGADSIDA

SEQ ID NO: 116 - protein, 104 aa, synthetic construct
  REGION 1..104: note = VL of anti-CD40L antibody (mouse)
LTQPSSVSANPGGTVEITCSGGYSDYYGWYQQKAPGSAPVTVIYYNDKRPSNIPSRFSGSTSGSTGTLTITGVQAEDEAIYYCGGYDGSTDAGIFGAGTTLTVL

SEQ ID NO: 117 - protein, 124 aa, synthetic construct
  REGION 1..124: note = VH of anti-CD40L antibody (mouse)
AVTLDESEGGLQTPGGALSLVCKASGFTFNNNGMAWVRQAPGKGLEFVAGISSGSYTYYGTAVKGRATISRDNGQSTVRLQLNNLRAEDTATYFCAKDGSDYNWNSGADSIDAWGHGTEVIVSS

SEQ ID NO: 118 - protein, 18 aa, synthetic construct
  REGION 1..18: note = peptide linker
GQSSRSSSGGGSSGGGGS

SEQ ID NO: 119 - protein, 648 aa, synthetic construct
  REGION 1..648: note = anti-CD40L/anti-CD28 bispecific antibody (mouse)
DIVMTQSPYSLAVSAGEKVTMSCRSSQSLYYSGIKKNLLAWYQQKPGQSPKLLIYFTSTRLPGVPDRFTGSGSGTDYTLTITSVQAEDMGHYFCQQGISTPLTFGDGTKLEIRGQSSRSSGGGGSSGGGGSQVQLKQSGAELVKPGASVKISCKTSGYTFTDGYMNWVEQKPGQGLEWIGRIDPDSGNTRYNQKFQGKATLTRDKSSSTVYMDLRSLTSEDSAVYYCARDGTFYGTYGYWYFDFWGQGTQVTVSSGQAGQGGGGSGGGGSGGGGSKLRTVAAPSVFIFPPSDEQLKSGTASVVCLLNNFYPREAKVQWKVDNALQSGNSQESVTEQDSKDSTYSLSSTLTLSKADYEKHKVYACEVTHQGLSLPVTKSFNRGESLEGGGGSGGGGSGGGGSTGLTQPSSVSANPGGTVEITCSGGYSDYYGWYQQKAPGSAPVTVIYYNDKRPSNIPSRFSGSTSGSTGTLTITGVQAEDEAIYYCGGYDGSTDAGIFGAGTTLTVLGQSSRSSSGGGSSGGGGSAVTLDESEGGLQTPGGALSLVCKAGFTFNNNGMAWVRQAPGKGLEFVAGISSGSYTYYGTAVKGRATISRDNGQSTVRLQLNNLRAEDTATYFCAKDGSDYNWNSGADSIDAWGHGTEVIVSS

SEQ ID NO: 120 - protein, 13 aa, synthetic construct
  REGION 1..13: note = L-CDR1 of anti-cotinine antibody
QSSQSPYSNEWLS

SEQ ID NO: 121 - protein, 7 aa, synthetic construct
  REGION 1..7: note = L-CDR2 of anti-cotinine antibody
RISTLAS

SEQ ID NO: 122 - protein, 12 aa, synthetic construct
  REGION 1..12: note = L-CDR3 of anti-cotinine antibody
AGGYNFGLFLFG

SEQ ID NO: 123 - protein, 5 aa, synthetic construct
  REGION 1..5: note = H-CDR1 of anti-cotinine antibody
RDWMN

SEQ ID NO: 124 - protein, 15 aa, synthetic construct
  REGION 1..15: note = H-CDR2 of anti-cotinine antibody
AIGRSGDTYYATWAK

SEQ ID NO: 125 - protein, 11 aa, synthetic construct
  REGION 1..11: note = H-CDR3 of anti-cotinine antibody
IPYFGWNNGDI

SEQ ID NO: 126 - protein, 110 aa, synthetic construct
  REGION 1..110: note = VL of anti-cotinine antibody
DIQMTQSPSSLSASVGDRVTITCQSSQSPYSNEWLSWYQQKPGKAPKLLIYRISTLASGVPSRFSGSRSGTDFTLTISSLQPEDFATYYCAGGYNFGLFLFGQGTKVEIK

SEQ ID NO: 127 - protein, 119 aa, synthetic construct
  REGION 1..119: note = VH of anti-cotinine antibody
EVQLVESGGGLVQPGGSLRLSCAASGHLRRRDWMNWVRQAPGKGLEWVAAIGRSGDTYYATWAKGRFTISADTSKNTAYLQMNSLRAEDTAVYYCSRIPYFGWNNGDIWGQGTLVTVSS

SEQ ID NO: 128 - protein, 108 aa, synthetic construct
  REGION 1..108: note = VL of anti-CD40L antibody
ELTQDPAVSVALGQTVRITCSGGYSSYGIYYYGWYQQKPGQAPVLVIYNGNKRPSGIPDRFSGSSSGNTASLTITGAQAEDEADYYCGSGDSSSDSGIFGGGTKLTVL